European Patent Specification EP 3 391 900 B1, published July 1, 2026. Title: PEPTIDES AND COMPOSITIONS FOR TREATMENT OF JOINT DAMAGE. Applicant: JOHNSON, Kristen SHI, Jian. The sequence listing filed with the application follows.

SEQUENCE LISTING (74 sequences)

SEQ ID NO: 1 - protein, 460 aa, Homo sapiens
MFTIKLLLFIVPLVISSRIDQDNSSFDSLSPEPKSRFAMLDDVKILANGLLQLGHGLKDFVHKTKGQINDIFQKLNIFDQSFYDLSLQTSEIKEEEKELRRTTYKLQVKNEEVKNMSLELNSKLESLLEEKILLQQKVKYLEEQLTNLIQNQPETPEHPEVTSLKTFVEKQDNSIKDLLQTVEDQYKQLNQQHSQIKEIENQLRRTSIQEPTEISLSSKPRAPRTTPFLQLNEIRNVKHDGIPAECTTIYNRGEHTSGMYAIRPSNSQVFHVYCDVISGSPWTLIQHRIDGSQNFNETWENYKYGFGRLDGEFWLGLEKIYSIVKQSNYVLRIELEDWKDNKHYIEYSFYLGNHETNYTLHLVAITGNVPNAIPENKDLVFSTWDHKAKGHFNCPEGYSGGWWWHDECGENNLNGKYNKPRAKSKPERRRGLSWKSQNGRLYSIKSTKMLIHPTDSESFE

SEQ ID NO: 2 - DNA, 2126 bp, Homo sapiens
ttccagaagaaaacagttccacgttgcttgaaattgaaaatcaagataaaaatgttcacaattaagctccttctttttattgttcctctagttatttcctccagaattgatcaagacaattcatcatttgattctctatctccagagccaaaatcaagatttgctatgttagacgatgtaaaaattttagccaatggcctccttcagttgggacatggtcttaaagactttgtccataagacgaagggccaaattaatgacatatttcaaaaactcaacatatttgatcagtctttttatgatctatcgctgcaaaccagtgaaatcaaagaagaagaaaaggaactgagaagaactacatataaactacaagtcaaaaatgaagaggtaaagaatatgtcacttgaactcaactcaaaacttgaaagcctcctagaagaaaaaattctacttcaacaaaaagtgaaatatttagaagagcaactaactaacttaattcaaaatcaacctgaaactccagaacacccagaagtaacttcacttaaaacttttgtagaaaaacaagataatagcatcaaagaccttctccagaccgtggaagaccaatataaacaattaaaccaacagcatagtcaaataaaagaaatagaaaatcagctcagaaggactagtattcaagaacccacagaaatttctctatcttccaagccaagagcaccaagaactactccctttcttcagttgaatgaaataagaaatgtaaaacatgatggcattcctgctgaatgtaccaccatttataacagaggtgaacatacaagtggcatgtatgccatcagacccagcaactctcaagtttttcatgtctactgtgatgttatatcaggtagtccatggacattaattcaacatcgaatagatggatcacaaaacttcaatgaaacgtgggagaactacaaatatggttttgggaggcttgatggagaattttggttgggcctagagaagatatactccatagtgaagcaatctaattatgttttacgaattgagttggaagactggaaagacaacaaacattatattgaatattctttttacttgggaaatcacgaaaccaactatacgctacatctagttgcgattactggcaatgtccccaatgcaatcccggaaaacaaagatttggtgttttctacttgggatcacaaagcaaaaggacacttcaactgtccagagggttattcaggaggctggtggtggcatgatgagtgtggagaaaacaacctaaatggtaaatataacaaaccaagagcaaaatctaagccagagaggagaagaggattatcttggaagtctcaaaatggaaggttatactctataaaatcaaccaaaatgttgatccatccaacagattcagaaagctttgaatgaactgaggcaaatttaaaaggcaataatttaaacattaacctcattccaagttaatgtggtctaataatctggtattaaatccttaagagaaagcttgagaaatagattttttttatcttaaagtcactgtctatttaagattaaacatacaatcacataaccttaaagaataccgtttacatttctcaatcaaaattcttataatactatttgttttaaattttgtgatgtgggaatcaattttagatggtcacaatctagattataatcaataggtgaacttattaaataacttttctaaataaaaaatttagagacttttattttaaaaggcatcatatgagctaatatcacaactttcccagtttaaaaaactagtactcttgttaaaactctaaacttgactaaatacagaggactggtaattgtacagttcttaaatgttgtagtattaatttcaaaactaaaaatcgtcagcacagagtatgtgtaaaaatctgtaatacaaatttttaaactgatgcttcattttgctacaaaataatttggagtaaatgtttgatatgatttatttatgaaacctaatgaagcagaattaaatactgtattaaaataagttcgctgtctttaaacaaatggagatgactactaagtcacattgactttaacatgaggtatcactataccttatt

SEQ ID NO: 3 - protein, 455 aa, Mus musculus
MHTIKLFLFVVPLVIASRVDPDLSSFDSAPSEPKSRFAMLDDVKILANGLLQLGHGLKDFVHKTKGQINDIFQKLNIFDQSFYDLSLRTNEIKEEEKELRRTTSTLQVKNEEVKNMSVELNSKLESLLEEKTALQHKVRALEEQLTNLILSPAGAQEHPEVTSLKSFVEQQDNSIRELLQSVEEQYKQLSQQHMQIKEIEKQLRKTGIQEPSENSLSSKSRAPRTTPPLQLNETENTEQDDLPADCSAVYNRGEHTSGVYTIKPRNSQGFNVYCDTQSGSPWTLIQHRKDGSQDFNETWENYEKGFGRLDGEFWLGLEKIYAIVQQSNYILRLELQDWKDSKHYVEYSFHLGSHETNYTLHVAEIAGNIPGALPEHTDLMFSTWNHRAKGQLYCPESYSGGWWWNDICGENNLNGKYNKPRTKSRPERRRGIYWRPQSRKLYAIKSSKMMLQPTT

SEQ ID NO: 4 - protein, 459 aa, Canis familiaris
MYTIKLFLFIIPLVISSKIDRDYSSYDSVSPEPKSRFAMLDDVKILANGLLQLGHGLKDFVHKTKGQINDIFQKLNIFDQSFYDLSLQTNEIKEEEKELRRTTSKLQVKNEEVKNMSLELNSKVESLLEEKILLQQKVRYLEKQLTSLIKNQPEIQEHPEVTSLKTFVEQQDNSIKDLLQTVEEQYRQLNQQHSQIKEIENQLRNVIQESTENSLSSKPRAPRTTPFLHLNETKNVEHNDIPANCTTIYNRGEHTSGIYSIRPSNSQVFNVYCDVKSGSSWTLIQHRIDGSQNFNETWENYRYGFGRLDGEFWLGLEKIYSIVKQSNYILRIELEDWNDNKHYIEYFFHLGNHETNYTLHLVEITGNILNALPEHKDLVFSTWDHKAKGHVNCPESYSGGWWWHNVCGENNLNGKYNKQRAKTKPERRRGLYWKSQNGRLYSIKSTKMLIHPIDSESSE

SEQ ID NO: 5 - protein, 469 aa, Equus caballus
MYTIKLFLVIAPLVISSRIDQDYSSLDSIPPEPKSRFAMLDDVKILANGLLQLGHGLKDFVHKTKGQINDIFQKLNIFDQSFYALSLQTNEIKEEEKELRRTTSKLQVKNEEVKNMSLELNSKLESLLEEKSLLQQKVKYLEEQLTKLIKNQPEIQEHPEVTSLKTFVEQQDNSIKDLLQTMEEQYRQLNQQHSQIKEIENQLRRTGIQESTENSLSSKPRAPRTTPSFHLNETKDVEHDDFPADCTTIYNRGEHTSGIYSIKPSNSQVFNVYCDVISGSSWILIQRRIDGSQNFNETWQNYKYGFGRLDFEFWLGLEKIYSIVKRSNYILRIELEDWKDNKHTIEYSFHLGNHETNYTLHLVEITGNVPNALPEHKDLVFSTWDHKAKGQLNCLESYSGGWWWHDVCGGDNPNGKYNKPRSKTKPERRRGICWKSQNGRLYTIKSTKMLIHPIDSESFELRQIKKPMN

SEQ ID NO: 6 - protein, 459 aa, Bos taurus
MYTIKLFLIIAPLVISSRTDQDYTSLDSISPEPKSRFAMLDDVKILANGLLQLGHGLKDFVHKTKGQINDIFQKLNIFDQSFYDLSLQTNEIKEEEKELRRATSKLQVKNEEVKNMSLELDSKLESLLEEKILLQQKVRYLEDQLTDLIKNQPQIQEYLEVTSLKTLVEQQDNSIKDLLQIVEEQYRQLNQQQSQIKEIENQLRRTGIKESTEISLSSKPRAPRTTPSFHSNETKNVEHDDIPADCTIIYNQGKHTSGIYSIRPSNSQVFNVYCDVKSGSSWTLIQHRIDGSQNFNETWENYKYGFGRLDGEFWLGLEKIYSIVMQSNYILRIELEDWKDKYYTEYSFHLGDHETNYTLHLAEISGNGPKAFPEHKDLMFSTWDHKAKGHFNCPESNSGGWWYHDVCGENNLNGKYNKPKAKAKPERKEGICWKSQDGRLYSIKATKMLIHPSDSENSE

SEQ ID NO: 7 - protein, 248 aa, Homo sapiens
IQEPTEISLSSKPRAPRTTPFLQLNEIRNVKHDGIPAECTTIYNRGEHTSGMYAIRPSNSQVFHVYCDVISGSPWTLIQHRIDGSQNFNETWENYKYGFGRLDGEFWLGLEKIYSIVKQSNYVLRIELEDWKDNKHYIEYSFYLGNHETNYTLHLVAITGNVPNAIPENKDLVFSTWDHKAKGHFNCPEGYSGGWWWHDECGENNLNGKYNKPRAKSKPERRRGLSWKSQNGRLYSIKSTKMLIHPTD

SEQ ID NO: 8 - protein, 231 aa, Homo sapiens
TTPFLQLNEIRNVKHDGIPAECTTIYNRGEHTSGMYAIRPSNSQVFHVYCDVISGSPWTLIQHRIDGSQNFNETWENYKYGFGRLDGEFWLGLEKIYSIVKQSNYVLRIELEDWKDNKHYIEYSFYLGNHETNYTLHLVAITGNVPNAIPENKDLVFSTWDHKAKGHFNCPEGYSGGWWWHDECGENNLNGKYNKPRAKSKPERRRGLSWKSQNGRLYSIKSTKMLIHPTD

SEQ ID NO: 9 - protein, 228 aa, Homo sapiens
FLQLNEIRNVKHDGIPAECTTIYNRGEHTSGMYAIRPSNSQVFHVYCDVISGSPWTLIQHRIDGSQNFNETWENYKYGFGRLDGEFWLGLEKIYSIVKQSNYVLRIELEDWKDNKHYIEYSFYLGNHETNYTLHLVAITGNVPNAIPENKDLVFSTWDHKAKGHFNCPEGYSGGWWWHDECGENNLNGKYNKPRAKSKPERRRGLSWKSQNGRLYSIKSTKMLIHPTD

SEQ ID NO: 10 - protein, 223 aa, Homo sapiens
EIRNVKHDGIPAECTTIYNRGEHTSGMYAIRPSNSQVFHVYCDVISGSPWTLIQHRIDGSQNFNETWENYKYGFGRLDGEFWLGLEKIYSIVKQSNYVLRIELEDWKDNKHYIEYSFYLGNHETNYTLHLVAITGNVPNAIPENKDLVFSTWDHKAKGHFNCPEGYSGGWWWHDECGENNLNGKYNKPRAKSKPERRRGLSWKSQNGRLYSIKSTKMLIHPTD

SEQ ID NO: 11 - protein, 215 aa, Homo sapiens
GIPAECTTIYNRGEHTSGMYAIRPSNSQVFHVYCDVISGSPWTLIQHRIDGSQNFNETWENYKYGFGRLDGEFWLGLEKIYSIVKQSNYVLRIELEDWKDNKHYIEYSFYLGNHETNYTLHLVAITGNVPNAIPENKDLVFSTWDHKAKGHFNCPEGYSGGWWWHDECGENNLNGKYNKPRAKSKPERRRGLSWKSQNGRLYSIKSTKMLIHPTD

SEQ ID NO: 12 - protein, 460 aa, Artificial Sequence
  K423Q
MFTIKLLLFIVPLVISSRIDQDNSSFDSLSPEPKSRFAMLDDVKILANGLLQLGHGLKDFVHKTKGQINDIFQKLNIFDQSFYDLSLQTSEIKEEEKELRRTTYKLQVKNEEVKNMSLELNSKLESLLEEKILLQQKVKYLEEQLTNLIQNQPETPEHPEVTSLKTFVEKQDNSIKDLLQTVEDQYKQLNQQHSQIKEIENQLRRTSIQEPTEISLSSKPRAPRTTPFLQLNEIRNVKHDGIPAECTTIYNRGEHTSGMYAIRPSNSQVFHVYCDVISGSPWTLIQHRIDGSQNFNETWENYKYGFGRLDGEFWLGLEKIYSIVKQSNYVLRIELEDWKDNKHYIEYSFYLGNHETNYTLHLVAITGNVPNAIPENKDLVFSTWDHKAKGHFNCPEGYSGGWWWHDECGENNLNGKYNKPRAQSKPERRRGLSWKSQNGRLYSIKSTKMLIHPTDSESFE

SEQ ID NO: 13 - protein, 460 aa, Artificial Sequence
  K423S
MFTIKLLLFIVPLVISSRIDQDNSSFDSLSPEPKSRFAMLDDVKILANGLLQLGHGLKDFVHKTKGQINDIFQKLNIFDQSFYDLSLQTSEIKEEEKELRRTTYKLQVKNEEVKNMSLELNSKLESLLEEKILLQQKVKYLEEQLTNLIQNQPETPEHPEVTSLKTFVEKQDNSIKDLLQTVEDQYKQLNQQHSQIKEIENQLRRTSIQEPTEISLSSKPRAPRTTPFLQLNEIRNVKHDGIPAECTTIYNRGEHTSGMYAIRPSNSQVFHVYCDVISGSPWTLIQHRIDGSQNFNETWENYKYGFGRLDGEFWLGLEKIYSIVKQSNYVLRIELEDWKDNKHYIEYSFYLGNHETNYTLHLVAITGNVPNAIPENKDLVFSTWDHKAKGHFNCPEGYSGGWWWHDECGENNLNGKYNKPRASSKPERRRGLSWKSQNGRLYSIKSTKMLIHPTDSESFE

SEQ ID NO: 14 - protein, 253 aa, Artificial Sequence
  207-460 K423Q
IQEPTEISLSSKPRAPRTTPFLQLNEIRNVKHDGIPAECTTIYNRGEHTSGMYAIRPSNSQVFHVYCDVISGSPWTLIQHRIDGSQNFNETWENYKYGFGRLDGEFWLGLEKIYSIVKQSNYVLRIELEDWKDNKHYIEYSFYLGNHETNYTLHLVAITGNVPNAIPENKDLVFSTWDHKAKGHFNCPEGYSGGWWWHDECGENNLNGKYNKPRAQSKPERRRGLSWKSQNGRLYSIKSTKMLIHPTDSESFE

SEQ ID NO: 15 - protein, 253 aa, Artificial Sequence
  207-460 K423S
IQEPTEISLSSKPRAPRTTPFLQLNEIRNVKHDGIPAECTTIYNRGEHTSGMYAIRPSNSQVFHVYCDVISGSPWTLIQHRIDGSQNFNETWENYKYGFGRLDGEFWLGLEKIYSIVKQSNYVLRIELEDWKDNKHYIEYSFYLGNHETNYTLHLVAITGNVPNAIPENKDLVFSTWDHKAKGHFNCPEGYSGGWWWHDECGENNLNGKYNKPRASSKPERRRGLSWKSQNGRLYSIKSTKMLIHPTDSESFE

SEQ ID NO: 16 - protein, 236 aa, Artificial Sequence
  225-460 K423Q
TTPFLQLNEIRNVKHDGIPAECTTIYNRGEHTSGMYAIRPSNSQVFHVYCDVISGSPWTLIQHRIDGSQNFNETWENYKYGFGRLDGEFWLGLEKIYSIVKQSNYVLRIELEDWKDNKHYIEYSFYLGNHETNYTLHLVAITGNVPNAIPENKDLVFSTWDHKAKGHFNCPEGYSGGWWWHDECGENNLNGKYNKPRAQSKPERRRGLSWKSQNGRLYSIKSTKMLIHPTDSESFE

SEQ ID NO: 17 - protein, 236 aa, Artificial Sequence
  225-460 K423S
TTPFLQLNEIRNVKHDGIPAECTTIYNRGEHTSGMYAIRPSNSQVFHVYCDVISGSPWTLIQHRIDGSQNFNETWENYKYGFGRLDGEFWLGLEKIYSIVKQSNYVLRIELEDWKDNKHYIEYSFYLGNHETNYTLHLVAITGNVPNAIPENKDLVFSTWDHKAKGHFNCPEGYSGGWWWHDECGENNLNGKYNKPRASSKPERRRGLSWKSQNGRLYSIKSTKMLIHPTDSESFE

SEQ ID NO: 18 - protein, 236 aa, Artificial Sequence
  225-460 S424T
TTPFLQLNEIRNVKHDGIPAECTTIYNRGEHTSGMYAIRPSNSQVFHVYCDVISGSPWTLIQHRIDGSQNFNETWENYKYGFGRLDGEFWLGLEKIYSIVKQSNYVLRIELEDWKDNKHYIEYSFYLGNHETNYTLHLVAITGNVPNAIPENKDLVFSTWDHKAKGHFNCPEGYSGGWWWHDECGENNLNGKYNKPRAKTKPERRRGLSWKSQNGRLYSIKSTKMLIHPTDSESFE

SEQ ID NO: 19 - protein, 235 aa, Artificial Sequence
  226-460 K423Q
TPFLQLNEIRNVKHDGIPAECTTIYNRGEHTSGMYAIRPSNSQVFHVYCDVISGSPWTLIQHRIDGSQNFNETWENYKYGFGRLDGEFWLGLEKIYSIVKQSNYVLRIELEDWKDNKHYIEYSFYLGNHETNYTLHLVAITGNVPNAIPENKDLVFSTWDHKAKGHFNCPEGYSGGWWWHDECGENNLNGKYNKPRAQSKPERRRGLSWKSQNGRLYSIKSTKMLIHPTDSESFE

SEQ ID NO: 20 - protein, 235 aa, Artificial Sequence
  226-460 K423S
TPFLQLNEIRNVKHDGIPAECTTIYNRGEHTSGMYAIRPSNSQVFHVYCDVISGSPWTLIQHRIDGSQNFNETWENYKYGFGRLDGEFWLGLEKIYSIVKQSNYVLRIELEDWKDNKHYIEYSFYLGNHETNYTLHLVAITGNVPNAIPENKDLVFSTWDHKAKGHFNCPEGYSGGWWWHDECGENNLNGKYNKPRASSKPERRRGLSWKSQNGRLYSIKSTKMLIHPTDSESFE

SEQ ID NO: 21 - protein, 233 aa, Artificial Sequence
  228-460 K423Q
FLQLNEIRNVKHDGIPAECTTIYNRGEHTSGMYAIRPSNSQVFHVYCDVISGSPWTLIQHRIDGSQNFNETWENYKYGFGRLDGEFWLGLEKIYSIVKQSNYVLRIELEDWKDNKHYIEYSFYLGNHETNYTLHLVAITGNVPNAIPENKDLVFSTWDHKAKGHFNCPEGYSGGWWWHDECGENNLNGKYNKPRAQSKPERRRGLSWKSQNGRLYSIKSTKMLIHPTDSESFE

SEQ ID NO: 22 - protein, 233 aa, Artificial Sequence
  228-460 K423S
FLQLNEIRNVKHDGIPAECTTIYNRGEHTSGMYAIRPSNSQVFHVYCDVISGSPWTLIQHRIDGSQNFNETWENYKYGFGRLDGEFWLGLEKIYSIVKQSNYVLRIELEDWKDNKHYIEYSFYLGNHETNYTLHLVAITGNVPNAIPENKDLVFSTWDHKAKGHFNCPEGYSGGWWWHDECGENNLNGKYNKPRASSKPERRRGLSWKSQNGRLYSIKSTKMLIHPTDSESFE

SEQ ID NO: 23 - protein, 233 aa, Artificial Sequence
  228-460 S424T
FLQLNEIRNVKHDGIPAECTTIYNRGEHTSGMYAIRPSNSQVFHVYCDVISGSPWTLIQHRIDGSQNFNETWENYKYGFGRLDGEFWLGLEKIYSIVKQSNYVLRIELEDWKDNKHYIEYSFYLGNHETNYTLHLVAITGNVPNAIPENKDLVFSTWDHKAKGHFNCPEGYSGGWWWHDECGENNLNGKYNKPRAKTKPERRRGLSWKSQNGRLYSIKSTKMLIHPTDSESFE

SEQ ID NO: 24 - protein, 228 aa, Artificial Sequence
  233-460 K423Q
EIRNVKHDGIPAECTTIYNRGEHTSGMYAIRPSNSQVFHVYCDVISGSPWTLIQHRIDGSQNFNETWENYKYGFGRLDGEFWLGLEKIYSIVKQSNYVLRIELEDWKDNKHYIEYSFYLGNHETNYTLHLVAITGNVPNAIPENKDLVFSTWDHKAKGHFNCPEGYSGGWWWHDECGENNLNGKYNKPRAQSKPERRRGLSWKSQNGRLYSIKSTKMLIHPTDSESFE

SEQ ID NO: 25 - protein, 228 aa, Artificial Sequence
  233-460 K423S
EIRNVKHDGIPAECTTIYNRGEHTSGMYAIRPSNSQVFHVYCDVISGSPWTLIQHRIDGSQNFNETWENYKYGFGRLDGEFWLGLEKIYSIVKQSNYVLRIELEDWKDNKHYIEYSFYLGNHETNYTLHLVAITGNVPNAIPENKDLVFSTWDHKAKGHFNCPEGYSGGWWWHDECGENNLNGKYNKPRASSKPERRRGLSWKSQNGRLYSIKSTKMLIHPTDSESFE

SEQ ID NO: 26 - protein, 220 aa, Artificial Sequence
  241-460 K423Q
GIPAECTTIYNRGEHTSGMYAIRPSNSQVFHVYCDVISGSPWTLIQHRIDGSQNFNETWENYKYGFGRLDGEFWLGLEKIYSIVKQSNYVLRIELEDWKDNKHYIEYSFYLGNHETNYTLHLVAITGNVPNAIPENKDLVFSTWDHKAKGHFNCPEGYSGGWWWHDECGENNLNGKYNKPRAQSKPERRRGLSWKSQNGRLYSIKSTKMLIHPTDSESFE

SEQ ID NO: 27 - protein, 220 aa, Artificial Sequence
  241-460 K423S
GIPAECTTIYNRGEHTSGMYAIRPSNSQVFHVYCDVISGSPWTLIQHRIDGSQNFNETWENYKYGFGRLDGEFWLGLEKIYSIVKQSNYVLRIELEDWKDNKHYIEYSFYLGNHETNYTLHLVAITGNVPNAIPENKDLVFSTWDHKAKGHFNCPEGYSGGWWWHDECGENNLNGKYNKPRASSKPERRRGLSWKSQNGRLYSIKSTKMLIHPTDSESFE

SEQ ID NO: 28 - protein, 219 aa, Artificial Sequence
  242-460 K423Q
IPAECTTIYNRGEHTSGMYAIRPSNSQVFHVYCDVISGSPWTLIQHRIDGSQNFNETWENYKYGFGRLDGEFWLGLEKIYSIVKQSNYVLRIELEDWKDNKHYIEYSFYLGNHETNYTLHLVAITGNVPNAIPENKDLVFSTWDHKAKGHFNCPEGYSGGWWWHDECGENNLNGKYNKPRAQSKPERRRGLSWKSQNGRLYSIKSTKMLIHPTDSESFE

SEQ ID NO: 29 - protein, 219 aa, Artificial Sequence
  242-460 K423S
IPAECTTIYNRGEHTSGMYAIRPSNSQVFHVYCDVISGSPWTLIQHRIDGSQNFNETWENYKYGFGRLDGEFWLGLEKIYSIVKQSNYVLRIELEDWKDNKHYIEYSFYLGNHETNYTLHLVAITGNVPNAIPENKDLVFSTWDHKAKGHFNCPEGYSGGWWWHDECGENNLNGKYNKPRASSKPERRRGLSWKSQNGRLYSIKSTKMLIHPTDSESFE

SEQ ID NO: 30 - protein, 231 aa, Artificial Sequence
  225-455 K423Q
TTPFLQLNEIRNVKHDGIPAECTTIYNRGEHTSGMYAIRPSNSQVFHVYCDVISGSPWTLIQHRIDGSQNFNETWENYKYGFGRLDGEFWLGLEKIYSIVKQSNYVLRIELEDWKDNKHYIEYSFYLGNHETNYTLHLVAITGNVPNAIPENKDLVFSTWDHKAKGHFNCPEGYSGGWWWHDECGENNLNGKYNKPRAQSKPERRRGLSWKSQNGRLYSIKSTKMLIHPTD

SEQ ID NO: 31 - protein, 231 aa, Artificial Sequence
  225-455 K423S
TTPFLQLNEIRNVKHDGIPAECTTIYNRGEHTSGMYAIRPSNSQVFHVYCDVISGSPWTLIQHRIDGSQNFNETWENYKYGFGRLDGEFWLGLEKIYSIVKQSNYVLRIELEDWKDNKHYIEYSFYLGNHETNYTLHLVAITGNVPNAIPENKDLVFSTWDHKAKGHFNCPEGYSGGWWWHDECGENNLNGKYNKPRASSKPERRRGLSWKSQNGRLYSIKSTKMLIHPTD

SEQ ID NO: 32 - protein, 230 aa, Artificial Sequence
  226-455 K423Q
TPFLQLNEIRNVKHDGIPAECTTIYNRGEHTSGMYAIRPSNSQVFHVYCDVISGSPWTLIQHRIDGSQNFNETWENYKYGFGRLDGEFWLGLEKIYSIVKQSNYVLRIELEDWKDNKHYIEYSFYLGNHETNYTLHLVAITGNVPNAIPENKDLVFSTWDHKAKGHFNCPEGYSGGWWWHDECGENNLNGKYNKPRAQSKPERRRGLSWKSQNGRLYSIKSTKMLIHPTD

SEQ ID NO: 33 - protein, 230 aa, Artificial Sequence
  226-455 K423S
TPFLQLNEIRNVKHDGIPAECTTIYNRGEHTSGMYAIRPSNSQVFHVYCDVISGSPWTLIQHRIDGSQNFNETWENYKYGFGRLDGEFWLGLEKIYSIVKQSNYVLRIELEDWKDNKHYIEYSFYLGNHETNYTLHLVAITGNVPNAIPENKDLVFSTWDHKAKGHFNCPEGYSGGWWWHDECGENNLNGKYNKPRASSKPERRRGLSWKSQNGRLYSIKSTKMLIHPTD

SEQ ID NO: 34 - protein, 228 aa, Artificial Sequence
  228-455 K423Q
FLQLNEIRNVKHDGIPAECTTIYNRGEHTSGMYAIRPSNSQVFHVYCDVISGSPWTLIQHRIDGSQNFNETWENYKYGFGRLDGEFWLGLEKIYSIVKQSNYVLRIELEDWKDNKHYIEYSFYLGNHETNYTLHLVAITGNVPNAIPENKDLVFSTWDHKAKGHFNCPEGYSGGWWWHDECGENNLNGKYNKPRAQSKPERRRGLSWKSQNGRLYSIKSTKMLIHPTD

SEQ ID NO: 35 - protein, 228 aa, Artificial Sequence
  228-455 K423S
FLQLNEIRNVKHDGIPAECTTIYNRGEHTSGMYAIRPSNSQVFHVYCDVISGSPWTLIQHRIDGSQNFNETWENYKYGFGRLDGEFWLGLEKIYSIVKQSNYVLRIELEDWKDNKHYIEYSFYLGNHETNYTLHLVAITGNVPNAIPENKDLVFSTWDHKAKGHFNCPEGYSGGWWWHDECGENNLNGKYNKPRASSKPERRRGLSWKSQNGRLYSIKSTKMLIHPTD

SEQ ID NO: 36 - protein, 223 aa, Artificial Sequence
  233-455 K423Q
EIRNVKHDGIPAECTTIYNRGEHTSGMYAIRPSNSQVFHVYCDVISGSPWTLIQHRIDGSQNFNETWENYKYGFGRLDGEFWLGLEKIYSIVKQSNYVLRIELEDWKDNKHYIEYSFYLGNHETNYTLHLVAITGNVPNAIPENKDLVFSTWDHKAKGHFNCPEGYSGGWWWHDECGENNLNGKYNKPRAQSKPERRRGLSWKSQNGRLYSIKSTKMLIHPTD

SEQ ID NO: 37 - protein, 223 aa, Artificial Sequence
  233-455 K423S
EIRNVKHDGIPAECTTIYNRGEHTSGMYAIRPSNSQVFHVYCDVISGSPWTLIQHRIDGSQNFNETWENYKYGFGRLDGEFWLGLEKIYSIVKQSNYVLRIELEDWKDNKHYIEYSFYLGNHETNYTLHLVAITGNVPNAIPENKDLVFSTWDHKAKGHFNCPEGYSGGWWWHDECGENNLNGKYNKPRASSKPERRRGLSWKSQNGRLYSIKSTKMLIHPTD

SEQ ID NO: 38 - protein, 215 aa, Artificial Sequence
  241-455 K423Q
GIPAECTTIYNRGEHTSGMYAIRPSNSQVFHVYCDVISGSPWTLIQHRIDGSQNFNETWENYKYGFGRLDGEFWLGLEKIYSIVKQSNYVLRIELEDWKDNKHYIEYSFYLGNHETNYTLHLVAITGNVPNAIPENKDLVFSTWDHKAKGHFNCPEGYSGGWWWHDECGENNLNGKYNKPRAQSKPERRRGLSWKSQNGRLYSIKSTKMLIHPTD

SEQ ID NO: 39 - protein, 215 aa, Artificial Sequence
  241-455 K423S
GIPAECTTIYNRGEHTSGMYAIRPSNSQVFHVYCDVISGSPWTLIQHRIDGSQNFNETWENYKYGFGRLDGEFWLGLEKIYSIVKQSNYVLRIELEDWKDNKHYIEYSFYLGNHETNYTLHLVAITGNVPNAIPENKDLVFSTWDHKAKGHFNCPEGYSGGWWWHDECGENNLNGKYNKPRASSKPERRRGLSWKSQNGRLYSIKSTKMLIHPTD

SEQ ID NO: 40 - protein, 214 aa, Artificial Sequence
  242-455 K423Q
IPAECTTIYNRGEHTSGMYAIRPSNSQVFHVYCDVISGSPWTLIQHRIDGSQNFNETWENYKYGFGRLDGEFWLGLEKIYSIVKQSNYVLRIELEDWKDNKHYIEYSFYLGNHETNYTLHLVAITGNVPNAIPENKDLVFSTWDHKAKGHFNCPEGYSGGWWWHDECGENNLNGKYNKPRAQSKPERRRGLSWKSQNGRLYSIKSTKMLIHPTD

SEQ ID NO: 41 - protein, 214 aa, Artificial Sequence
  242-455 K423S
IPAECTTIYNRGEHTSGMYAIRPSNSQVFHVYCDVISGSPWTLIQHRIDGSQNFNETWENYKYGFGRLDGEFWLGLEKIYSIVKQSNYVLRIELEDWKDNKHYIEYSFYLGNHETNYTLHLVAITGNVPNAIPENKDLVFSTWDHKAKGHFNCPEGYSGGWWWHDECGENNLNGKYNKPRASSKPERRRGLSWKSQNGRLYSIKSTKMLIHPTD

SEQ ID NO: 42 - protein, 233 aa, Artificial Sequence
  canine 227 K423Q
FLHLNETKNVEHNDIPANCTTIYNRGEHTSGIYSIRPSNSQVFNVYCDVKSGSSWTLIQHRIDGSQNFNETWENYRYGFGRLDGEFWLGLEKIYSIVKQSNYILRIELEDWNDNKHYIEYFFHLGNHETNYTLHLVEITGNILNALPEHKDLVFSTWDHKAKGHVNCPESYSGGWWWHNVCGENNLNGKYNKQRAQTKPERRRGLYWKSQNGRLYSIKSTKMLIHPIDSESSE

SEQ ID NO: 43 - protein, 233 aa, Artificial Sequence
  canine 227 K423S
FLHLNETKNVEHNDIPANCTTIYNRGEHTSGIYSIRPSNSQVFNVYCDVKSGSSWTLIQHRIDGSQNFNETWENYRYGFGRLDGEFWLGLEKIYSIVKQSNYILRIELEDWNDNKHYIEYFFHLGNHETNYTLHLVEITGNILNALPEHKDLVFSTWDHKAKGHVNCPESYSGGWWWHNVCGENNLNGKYNKQRASTKPERRRGLYWKSQNGRLYSIKSTKMLIHPIDSESSE

SEQ ID NO: 44 - DNA, 708 bp, Artificial Sequence
  nucleic acid encoding 225WT
actactccctttcttcagttgaatgaaataagaaatgtaaaacatgatggcattcctgctgaatgtaccaccatttataacagaggtgaacatacaagtggcatgtatgccatcagacccagcaactctcaagtttttcatgtctactgtgatgttatatcaggtagtccatggacattaattcaacatcgaatagatggatcacaaaacttcaatgaaacgtgggagaactacaaatatggttttgggaggcttgatggagaattttggttgggcctagagaagatatactccatagtgaagcaatctaattatgttttacgaattgagttggaagactggaaagacaacaaacattatattgaatattctttttacttgggaaatcacgaaaccaactatacgctacatctagttgcgattactggcaatgtccccaatgcaatcccggaaaacaaagatttggtgttttctacttgggatcacaaagcaaaaggacacttcaactgtccagagggttattcaggaggctggtggtggcatgatgagtgtggagaaaacaacctaaatggtaaatataacaaaccaagagcaaaatctaagccagagaggagaagaggattatcttggaagtctcaaaatggaaggttatactctataaaatcaaccaaaatgttgatccatccaacagattcagaaagctttgaa

SEQ ID NO: 45 - DNA, 708 bp, Artificial Sequence
  nucleic acid encoding 225 K423Q
actactccctttcttcagttgaatgaaataagaaatgtaaaacatgatggcattcctgctgaatgtaccaccatttataacagaggtgaacatacaagtggcatgtatgccatcagacccagcaactctcaagtttttcatgtctactgtgatgttatatcaggtagtccatggacattaattcaacatcgaatagatggatcacaaaacttcaatgaaacgtgggagaactacaaatatggttttgggaggcttgatggagaattttggttgggcctagagaagatatactccatagtgaagcaatctaattatgttttacgaattgagttggaagactggaaagacaacaaacattatattgaatattctttttacttgggaaatcacgaaaccaactatacgctacatctagttgcgattactggcaatgtccccaatgcaatcccggaaaacaaagatttggtgttttctacttgggatcacaaagcaaaaggacacttcaactgtccagagggttattcaggaggctggtggtggcatgatgagtgtggagaaaacaacctaaatggtaaatataacaaaccaagagcacaatctaagccagagaggagaagaggattatcttggaagtctcaaaatggaaggttatactctataaaatcaaccaaaatgttgatccatccaacagattcagaaagctttgaa

SEQ ID NO: 46 - DNA, 708 bp, Artificial Sequence
  nucleic acid encoding 225 K423S
actactccctttcttcagttgaatgaaataagaaatgtaaaacatgatggcattcctgctgaatgtaccaccatttataacagaggtgaacatacaagtggcatgtatgccatcagacccagcaactctcaagtttttcatgtctactgtgatgttatatcaggtagtccatggacattaattcaacatcgaatagatggatcacaaaacttcaatgaaacgtgggagaactacaaatatggttttgggaggcttgatggagaattttggttgggcctagagaagatatactccatagtgaagcaatctaattatgttttacgaattgagttggaagactggaaagacaacaaacattatattgaatattctttttacttgggaaatcacgaaaccaactatacgctacatctagttgcgattactggcaatgtccccaatgcaatcccggaaaacaaagatttggtgttttctacttgggatcacaaagcaaaaggacacttcaactgtccagagggttattcaggaggctggtggtggcatgatgagtgtggagaaaacaacctaaatggtaaatataacaaaccaagagcaagctctaagccagagaggagaagaggattatcttggaagtctcaaaatggaaggttatactctataaaatcaaccaaaatgttgatccatccaacagattcagaaagctttgaa

SEQ ID NO: 47 - DNA, 705 bp, Artificial Sequence
  nucleic acid encoding 226 K423Q
actccctttcttcagttgaatgaaataagaaatgtaaaacatgatggcattcctgctgaatgtaccaccatttataacagaggtgaacatacaagtggcatgtatgccatcagacccagcaactctcaagtttttcatgtctactgtgatgttatatcaggtagtccatggacattaattcaacatcgaatagatggatcacaaaacttcaatgaaacgtgggagaactacaaatatggttttgggaggcttgatggagaattttggttgggcctagagaagatatactccatagtgaagcaatctaattatgttttacgaattgagttggaagactggaaagacaacaaacattatattgaatattctttttacttgggaaatcacgaaaccaactatacgctacatctagttgcgattactggcaatgtccccaatgcaatcccggaaaacaaagatttggtgttttctacttgggatcacaaagcaaaaggacacttcaactgtccagagggttattcaggaggctggtggtggcatgatgagtgtggagaaaacaacctaaatggtaaatataacaaaccaagagcacaatctaagccagagaggagaagaggattatcttggaagtctcaaaatggaaggttatactctataaaatcaaccaaaatgttgatccatccaacagattcagaaagctttgaa

SEQ ID NO: 48 - DNA, 705 bp, Artificial Sequence
  nucleic acid encoding 226 K423S
actccctttcttcagttgaatgaaataagaaatgtaaaacatgatggcattcctgctgaatgtaccaccatttataacagaggtgaacatacaagtggcatgtatgccatcagacccagcaactctcaagtttttcatgtctactgtgatgttatatcaggtagtccatggacattaattcaacatcgaatagatggatcacaaaacttcaatgaaacgtgggagaactacaaatatggttttgggaggcttgatggagaattttggttgggcctagagaagatatactccatagtgaagcaatctaattatgttttacgaattgagttggaagactggaaagacaacaaacattatattgaatattctttttacttgggaaatcacgaaaccaactatacgctacatctagttgcgattactggcaatgtccccaatgcaatcccggaaaacaaagatttggtgttttctacttgggatcacaaagcaaaaggacacttcaactgtccagagggttattcaggaggctggtggtggcatgatgagtgtggagaaaacaacctaaatggtaaatataacaaaccaagagcaagctctaagccagagaggagaagaggattatcttggaagtctcaaaatggaaggttatactctataaaatcaaccaaaatgttgatccatccaacagattcagaaagctttgaa

SEQ ID NO: 49 - DNA, 699 bp, Artificial Sequence
  nucleic acid encoding 228 K423Q
tttcttcagttgaatgaaataagaaatgtaaaacatgatggcattcctgctgaatgtaccaccatttataacagaggtgaacatacaagtggcatgtatgccatcagacccagcaactctcaagtttttcatgtctactgtgatgttatatcaggtagtccatggacattaattcaacatcgaatagatggatcacaaaacttcaatgaaacgtgggagaactacaaatatggttttgggaggcttgatggagaattttggttgggcctagagaagatatactccatagtgaagcaatctaattatgttttacgaattgagttggaagactggaaagacaacaaacattatattgaatattctttttacttgggaaatcacgaaaccaactatacgctacatctagttgcgattactggcaatgtccccaatgcaatcccggaaaacaaagatttggtgttttctacttgggatcacaaagcaaaaggacacttcaactgtccagagggttattcaggaggctggtggtggcatgatgagtgtggagaaaacaacctaaatggtaaatataacaaaccaagagcacaatctaagccagagaggagaagaggattatcttggaagtctcaaaatggaaggttatactctataaaatcaaccaaaatgttgatccatccaacagattcagaaagctttgaa

SEQ ID NO: 50 - DNA, 699 bp, Artificial Sequence
  nucleic acid encoding 228 K423S
tttcttcagttgaatgaaataagaaatgtaaaacatgatggcattcctgctgaatgtaccaccatttataacagaggtgaacatacaagtggcatgtatgccatcagacccagcaactctcaagtttttcatgtctactgtgatgttatatcaggtagtccatggacattaattcaacatcgaatagatggatcacaaaacttcaatgaaacgtgggagaactacaaatatggttttgggaggcttgatggagaattttggttgggcctagagaagatatactccatagtgaagcaatctaattatgttttacgaattgagttggaagactggaaagacaacaaacattatattgaatattctttttacttgggaaatcacgaaaccaactatacgctacatctagttgcgattactggcaatgtccccaatgcaatcccggaaaacaaagatttggtgttttctacttgggatcacaaagcaaaaggacacttcaactgtccagagggttattcaggaggctggtggtggcatgatgagtgtggagaaaacaacctaaatggtaaatataacaaaccaagagcaagctctaagccagagaggagaagaggattatcttggaagtctcaaaatggaaggttatactctataaaatcaaccaaaatgttgatccatccaacagattcagaaagctttgaa

SEQ ID NO: 51 - DNA, 684 bp, Artificial Sequence
  nucleic acid encoding 233 K423Q
gaaataagaaatgtaaaacatgatggcattcctgctgaatgtaccaccatttataacagaggtgaacatacaagtggcatgtatgccatcagacccagcaactctcaagtttttcatgtctactgtgatgttatatcaggtagtccatggacattaattcaacatcgaatagatggatcacaaaacttcaatgaaacgtgggagaactacaaatatggttttgggaggcttgatggagaattttggttgggcctagagaagatatactccatagtgaagcaatctaattatgttttacgaattgagttggaagactggaaagacaacaaacattatattgaatattctttttacttgggaaatcacgaaaccaactatacgctacatctagttgcgattactggcaatgtccccaatgcaatcccggaaaacaaagatttggtgttttctacttgggatcacaaagcaaaaggacacttcaactgtccagagggttattcaggaggctggtggtggcatgatgagtgtggagaaaacaacctaaatggtaaatataacaaaccaagagcacaatctaagccagagaggagaagaggattatcttggaagtctcaaaatggaaggttatactctataaaatcaaccaaaatgttgatccatccaacagattcagaaagctttgaa

SEQ ID NO: 52 - DNA, 684 bp, Artificial Sequence
  nucleic acid encoding 233 K423S
gaaataagaaatgtaaaacatgatggcattcctgctgaatgtaccaccatttataacagaggtgaacatacaagtggcatgtatgccatcagacccagcaactctcaagtttttcatgtctactgtgatgttatatcaggtagtccatggacattaattcaacatcgaatagatggatcacaaaacttcaatgaaacgtgggagaactacaaatatggttttgggaggcttgatggagaattttggttgggcctagagaagatatactccatagtgaagcaatctaattatgttttacgaattgagttggaagactggaaagacaacaaacattatattgaatattctttttacttgggaaatcacgaaaccaactatacgctacatctagttgcgattactggcaatgtccccaatgcaatcccggaaaacaaagatttggtgttttctacttgggatcacaaagcaaaaggacacttcaactgtccagagggttattcaggaggctggtggtggcatgatgagtgtggagaaaacaacctaaatggtaaatataacaaaccaagagcaagctctaagccagagaggagaagaggattatcttggaagtctcaaaatggaaggttatactctataaaatcaaccaaaatgttgatccatccaacagattcagaaagctttgaa

SEQ ID NO: 53 - DNA, 660 bp, Artificial Sequence
  nucleic acid encoding 241 K423Q
ggcattcctgctgaatgtaccaccatttataacagaggtgaacatacaagtggcatgtatgccatcagacccagcaactctcaagtttttcatgtctactgtgatgttatatcaggtagtccatggacattaattcaacatcgaatagatggatcacaaaacttcaatgaaacgtgggagaactacaaatatggttttgggaggcttgatggagaattttggttgggcctagagaagatatactccatagtgaagcaatctaattatgttttacgaattgagttggaagactggaaagacaacaaacattatattgaatattctttttacttgggaaatcacgaaaccaactatacgctacatctagttgcgattactggcaatgtccccaatgcaatcccggaaaacaaagatttggtgttttctacttgggatcacaaagcaaaaggacacttcaactgtccagagggttattcaggaggctggtggtggcatgatgagtgtggagaaaacaacctaaatggtaaatataacaaaccaagagcacaatctaagccagagaggagaagaggattatcttggaagtctcaaaatggaaggttatactctataaaatcaaccaaaatgttgatccatccaacagattcagaaagctttgaa

SEQ ID NO: 54 - DNA, 660 bp, Artificial Sequence
  nucleic acid encoding 241 K423S
ggcattcctgctgaatgtaccaccatttataacagaggtgaacatacaagtggcatgtatgccatcagacccagcaactctcaagtttttcatgtctactgtgatgttatatcaggtagtccatggacattaattcaacatcgaatagatggatcacaaaacttcaatgaaacgtgggagaactacaaatatggttttgggaggcttgatggagaattttggttgggcctagagaagatatactccatagtgaagcaatctaattatgttttacgaattgagttggaagactggaaagacaacaaacattatattgaatattctttttacttgggaaatcacgaaaccaactatacgctacatctagttgcgattactggcaatgtccccaatgcaatcccggaaaacaaagatttggtgttttctacttgggatcacaaagcaaaaggacacttcaactgtccagagggttattcaggaggctggtggtggcatgatgagtgtggagaaaacaacctaaatggtaaatataacaaaccaagagcaagctctaagccagagaggagaagaggattatcttggaagtctcaaaatggaaggttatactctataaaatcaaccaaaatgttgatccatccaacagattcagaaagctttgaa

SEQ ID NO: 55 - DNA, 657 bp, Artificial Sequence
  nucleic acid encoding 242 K423Q
attcctgctgaatgtaccaccatttataacagaggtgaacatacaagtggcatgtatgccatcagacccagcaactctcaagtttttcatgtctactgtgatgttatatcaggtagtccatggacattaattcaacatcgaatagatggatcacaaaacttcaatgaaacgtgggagaactacaaatatggttttgggaggcttgatggagaattttggttgggcctagagaagatatactccatagtgaagcaatctaattatgttttacgaattgagttggaagactggaaagacaacaaacattatattgaatattctttttacttgggaaatcacgaaaccaactatacgctacatctagttgcgattactggcaatgtccccaatgcaatcccggaaaacaaagatttggtgttttctacttgggatcacaaagcaaaaggacacttcaactgtccagagggttattcaggaggctggtggtggcatgatgagtgtggagaaaacaacctaaatggtaaatataacaaaccaagagcacaatctaagccagagaggagaagaggattatcttggaagtctcaaaatggaaggttatactctataaaatcaaccaaaatgttgatccatccaacagattcagaaagctttgaa

SEQ ID NO: 56 - DNA, 657 bp, Artificial Sequence
  nucleic acid encoding 242 K423S
attcctgctgaatgtaccaccatttataacagaggtgaacatacaagtggcatgtatgccatcagacccagcaactctcaagtttttcatgtctactgtgatgttatatcaggtagtccatggacattaattcaacatcgaatagatggatcacaaaacttcaatgaaacgtgggagaactacaaatatggttttgggaggcttgatggagaattttggttgggcctagagaagatatactccatagtgaagcaatctaattatgttttacgaattgagttggaagactggaaagacaacaaacattatattgaatattctttttacttgggaaatcacgaaaccaactatacgctacatctagttgcgattactggcaatgtccccaatgcaatcccggaaaacaaagatttggtgttttctacttgggatcacaaagcaaaaggacacttcaactgtccagagggttattcaggaggctggtggtggcatgatgagtgtggagaaaacaacctaaatggtaaatataacaaaccaagagcaagctctaagccagagaggagaagaggattatcttggaagtctcaaaatggaaggttatactctataaaatcaaccaaaatgttgatccatccaacagattcagaaagctttgaa

SEQ ID NO: 57 - DNA, 699 bp, Artificial Sequence
  nucleic acid sequence encoding canine 227KQ
tttttgcatctcaacgaaacgaagaatgtcgaacacaacgacattccggcaaattgcacaactatctacaatagaggcgaacatacgtccggtatctactccattagaccttcaaacagccaggtattcaatgtgtactgcgatgtaaagtcaggatcgtcatggacactgatccagcataggatcgacgggtcccagaacttcaacgagacatgggagaactaccgctatggatttggaaggctggatggggagttctggttgggacttgagaaaatctacagcattgtgaagcagtcgaactacattctccggattgaactggaggactggaatgacaacaaacactacatcgagtatttctttcatctcggcaaccatgaaacgaattacaccttgcaccttgtggaaatcacgggcaacattttgaacgcgctgccagaacacaaagacctggtgttttcgacatgggatcacaaagcaaaggggcacgtgaactgtcccgaatcatatagcgggggatggtggtggcacaatgtctgtggtgagaacaatctcaacgggaaatacaataagcagcgagctcagacgaaacccgagcggcggagaggtctgtattggaagtcgcagaatggacgcctgtattcgatcaaatcgacgaaaatgctcatccaccccatcgactccgaatcgtcggag

SEQ ID NO: 58 - protein, 252 aa, Artificial Sequence
  201-460 K423del
IQEPTEISLSSKPRAPRTTPFLQLNEIRNVKHDGIPAECTTIYNRGEHTSGMYAIRPSNSQVFHVYCDVISGSPWTLIQHRIDGSQNFNETWENYKYGFGRLDGEFWLGLEKIYSIVKQSNYVLRIELEDWKDNKHYIEYSFYLGNHETNYTLHLVAITGNVPNAIPENKDLVFSTWDHKAKGHFNCPEGYSGGWWWHDECGENNLNGKYNKPRASKPERRRGLSWKSQNGRLYSIKSTKMLIHPTDSESFE

SEQ ID NO: 59 - protein, 235 aa, Artificial Sequence
  225-460 K423del
TTPFLQLNEIRNVKHDGIPAECTTIYNRGEHTSGMYAIRPSNSQVFHVYCDVISGSPWTLIQHRIDGSQNFNETWENYKYGFGRLDGEFWLGLEKIYSIVKQSNYVLRIELEDWKDNKHYIEYSFYLGNHETNYTLHLVAITGNVPNAIPENKDLVFSTWDHKAKGHFNCPEGYSGGWWWHDECGENNLNGKYNKPRASKPERRRGLSWKSQNGRLYSIKSTKMLIHPTDSESFE

SEQ ID NO: 60 - protein, 234 aa, Artificial Sequence
  226-460 K423del
TPFLQLNEIRNVKHDGIPAECTTIYNRGEHTSGMYAIRPSNSQVFHVYCDVISGSPWTLIQHRIDGSQNFNETWENYKYGFGRLDGEFWLGLEKIYSIVKQSNYVLRIELEDWKDNKHYIEYSFYLGNHETNYTLHLVAITGNVPNAIPENKDLVFSTWDHKAKGHFNCPEGYSGGWWWHDECGENNLNGKYNKPRASKPERRRGLSWKSQNGRLYSIKSTKMLIHPTDSESFE

SEQ ID NO: 61 - protein, 232 aa, Artificial Sequence
  228-460 K423del
FLQLNEIRNVKHDGIPAECTTIYNRGEHTSGMYAIRPSNSQVFHVYCDVISGSPWTLIQHRIDGSQNFNETWENYKYGFGRLDGEFWLGLEKIYSIVKQSNYVLRIELEDWKDNKHYIEYSFYLGNHETNYTLHLVAITGNVPNAIPENKDLVFSTWDHKAKGHFNCPEGYSGGWWWHDECGENNLNGKYNKPRASKPERRRGLSWKSQNGRLYSIKSTKMLIHPTDSESFE

SEQ ID NO: 62 - protein, 227 aa, Artificial Sequence
  233-460 K423del
EIRNVKHDGIPAECTTIYNRGEHTSGMYAIRPSNSQVFHVYCDVISGSPWTLIQHRIDGSQNFNETWENYKYGFGRLDGEFWLGLEKIYSIVKQSNYVLRIELEDWKDNKHYIEYSFYLGNHETNYTLHLVAITGNVPNAIPENKDLVFSTWDHKAKGHFNCPEGYSGGWWWHDECGENNLNGKYNKPRASKPERRRGLSWKSQNGRLYSIKSTKMLIHPTDSESFE

SEQ ID NO: 63 - protein, 219 aa, Artificial Sequence
  241-460 K423del
GIPAECTTIYNRGEHTSGMYAIRPSNSQVFHVYCDVISGSPWTLIQHRIDGSQNFNETWENYKYGFGRLDGEFWLGLEKIYSIVKQSNYVLRIELEDWKDNKHYIEYSFYLGNHETNYTLHLVAITGNVPNAIPENKDLVFSTWDHKAKGHFNCPEGYSGGWWWHDECGENNLNGKYNKPRASKPERRRGLSWKSQNGRLYSIKSTKMLIHPTDSESFE

SEQ ID NO: 64 - protein, 218 aa, Artificial Sequence
  242-460 K423del
IPAECTTIYNRGEHTSGMYAIRPSNSQVFHVYCDVISGSPWTLIQHRIDGSQNFNETWENYKYGFGRLDGEFWLGLEKIYSIVKQSNYVLRIELEDWKDNKHYIEYSFYLGNHETNYTLHLVAITGNVPNAIPENKDLVFSTWDHKAKGHFNCPEGYSGGWWWHDECGENNLNGKYNKPRASKPERRRGLSWKSQNGRLYSIKSTKMLIHPTDSESFE

SEQ ID NO: 65 - protein, 230 aa, Artificial Sequence
  225-455 K423del
TTPFLQLNEIRNVKHDGIPAECTTIYNRGEHTSGMYAIRPSNSQVFHVYCDVISGSPWTLIQHRIDGSQNFNETWENYKYGFGRLDGEFWLGLEKIYSIVKQSNYVLRIELEDWKDNKHYIEYSFYLGNHETNYTLHLVAITGNVPNAIPENKDLVFSTWDHKAKGHFNCPEGYSGGWWWHDECGENNLNGKYNKPRASKPERRRGLSWKSQNGRLYSIKSTKMLIHPTD

SEQ ID NO: 66 - protein, 229 aa, Artificial Sequence
  226-455 K423del
TPFLQLNEIRNVKHDGIPAECTTIYNRGEHTSGMYAIRPSNSQVFHVYCDVISGSPWTLIQHRIDGSQNFNETWENYKYGFGRLDGEFWLGLEKIYSIVKQSNYVLRIELEDWKDNKHYIEYSFYLGNHETNYTLHLVAITGNVPNAIPENKDLVFSTWDHKAKGHFNCPEGYSGGWWWHDECGENNLNGKYNKPRASKPERRRGLSWKSQNGRLYSIKSTKMLIHPTD

SEQ ID NO: 67 - protein, 227 aa, Artificial Sequence
  228-455 K423del
FLQLNEIRNVKHDGIPAECTTIYNRGEHTSGMYAIRPSNSQVFHVYCDVISGSPWTLIQHRIDGSQNFNETWENYKYGFGRLDGEFWLGLEKIYSIVKQSNYVLRIELEDWKDNKHYIEYSFYLGNHETNYTLHLVAITGNVPNAIPENKDLVFSTWDHKAKGHFNCPEGYSGGWWWHDECGENNLNGKYNKPRASKPERRRGLSWKSQNGRLYSIKSTKMLIHPTD

SEQ ID NO: 68 - protein, 222 aa, Artificial Sequence
  233-455 K423del
EIRNVKHDGIPAECTTIYNRGEHTSGMYAIRPSNSQVFHVYCDVISGSPWTLIQHRIDGSQNFNETWENYKYGFGRLDGEFWLGLEKIYSIVKQSNYVLRIELEDWKDNKHYIEYSFYLGNHETNYTLHLVAITGNVPNAIPENKDLVFSTWDHKAKGHFNCPEGYSGGWWWHDECGENNLNGKYNKPRASKPERRRGLSWKSQNGRLYSIKSTKMLIHPTD

SEQ ID NO: 69 - protein, 214 aa, Artificial Sequence
  241-455 K423del
GIPAECTTIYNRGEHTSGMYAIRPSNSQVFHVYCDVISGSPWTLIQHRIDGSQNFNETWENYKYGFGRLDGEFWLGLEKIYSIVKQSNYVLRIELEDWKDNKHYIEYSFYLGNHETNYTLHLVAITGNVPNAIPENKDLVFSTWDHKAKGHFNCPEGYSGGWWWHDECGENNLNGKYNKPRASKPERRRGLSWKSQNGRLYSIKSTKMLIHPTD

SEQ ID NO: 70 - protein, 213 aa, Artificial Sequence
  242-455 K423del
IPAECTTIYNRGEHTSGMYAIRPSNSQVFHVYCDVISGSPWTLIQHRIDGSQNFNETWENYKYGFGRLDGEFWLGLEKIYSIVKQSNYVLRIELEDWKDNKHYIEYSFYLGNHETNYTLHLVAITGNVPNAIPENKDLVFSTWDHKAKGHFNCPEGYSGGWWWHDECGENNLNGKYNKPRASKPERRRGLSWKSQNGRLYSIKSTKMLIHPTD

SEQ ID NO: 71 - protein, 491 aa, Homo sapiens
MKTFTWTLGVLFFLLVDTGHCRGGQFKIKKINQRRYPRATDGKEEAKKCAYTFLVPEQRITGPICVNTKGQDASTIKDMITRMDLENLKDVLSRQKREIDVLQLVVDVDGNIVNEVKLLRKESRNMNSRVTQLYMQLLHEIIRKRDNSLELSQLENKILNVTTEMLKMATRYRELEVKYASLTDLVNNQSVMITLLEEQCLRIFSRQDTHVSPPLVQVVPQHIPNSQQYTPGLLGGNEIQRDPGYPRDLMPPPDLATSPTKSPFKIPPVTFINEGPFKDCQQAKEAGHSVSGIYMIKPENSNGPMQLWCENSLDPGGWTVIQKRTDGSVNFFRNWENYKKGFGNIDGEYWLGLENIYMLSNQDNYKLLIELEDWSDKKVYAEYSSFRLEPESEFYRLRLGTYQGNAGDSMMWHNGKQFTTLDRDKDMYAGNCAHFHKGGWWYNACAHSNLNGVWYRGGHYRSKHQDGIFWAEYRGGSYSLRAVQMMIKPID

SEQ ID NO: 72 - protein, 221 aa, Artificial Sequence
  Cterminal hANGPTL1 271-491
FINEGPFKDCQQAKEAGHSVSGIYMIKPENSNGPMQLWCENSLDPGGWTVIQKRTDGSVNFFRNWENYKKGFGNIDGEYWLGLENIYMLSNQDNYKLLIELEDWSDKKVYAEYSSFRLEPESEFYRLRLGTYQGNAGDSMMWHNGKQFTTLDRDKDMYAGNCAHFHKGGWWYNACAHSNLNGVWYRGGHYRSKHQDGIFWAEYRGGSYSLRAVQMMIKPID

SEQ ID NO: 73 - protein, 406 aa, Homo sapiens
MSGAPTAGAALMLCAATAVLLSAQGGPVQSKSPRFASWDEMNVLAHGLLQLGQGLREHAERTRSQLSALERRLSACGSACQGTEGSTDLPLAPESRVDPEVLHSLQTQLKAQNSRIQQLFHKVAQQQRHLEKQHLRIQHLQSQFGLLDHKHLDHEVAKPARRKRLPEMAQPVDPAHNVSRLHRLPRDCQELFQVGERQSGLFEIQPQGSPPFLVNCKMTSDGGWTVIQRRHDGSVDFNRPWEAYKAGFGDPHGEFWLGLEKVHSITGDRNSRLAVQLRDWDGNAELLQFSVHLGGEDTAYSLQLTAPVAGQLGATTVPPSGLSVPFSTWDQDHDLRRDKNCAKSLSGGWWFGTCSHSNLNGQYFRSIPQQRQKLKKGIFWKTWRGRYYPLQATTMLIQPMAAEAAS

SEQ ID NO: 74 - protein, 228 aa, Artificial Sequence
  Cterminal hANGPTL4 179-406
SRLHRLPRDCQELFQVGERQSGLFEIQPQGSPPFLVNCKMTSDGGWTVIQRRHDGSVDFNRPWEAYKAGFGDPHGEFWLGLEKVHSITGDRNSRLAVQLRDWDGNAELLQFSVHLGGEDTAYSLQLTAPVAGQLGATTVPPSGLSVPFSTWDQDHDLRRDKNCAKSLSGGWWFGTCSHSNLNGQYFRSIPQQRQKLKKGIFWKTWRGRYYPLQATTMLIQPMAAEAAS